European Patent Application EP 4 238 996 A2, published September 6, 2023. Title: Antiviral antibody against SARS-CoV2 binding to ACE2 and uses thereof. Applicant: Daegu Gyeongbuk Institute of Science and Technology. The sequence listing filed with the application follows.

SEQUENCE LISTING (24 sequences)

SEQ ID NO: 1 - protein, 110 aa, Artificial Sequence
  C3-LC
QSVLTQPPSVSGAPGQRVTISCTGSSSNIGADYDVHWYQQLPGTAPKLLIYGNTNRPSGVPDRFSGSKSGTSASLAITGLQAEDEANYYCQSYESGLGWLFGGGTQLTVL

SEQ ID NO: 2 - protein, 121 aa, Artificial Sequence
  C3-HC
QVQLVESGGGLVQPGGSLRLSCAASGFTFSSYAMSWVRQAPGKGLEWVSAISGSGGSTYYADSVKGRFTISRDNSKNTLYLQMNSLRAEDTAVYYCAKYGRGLPPGHFDYWGQGTLVTVSS

SEQ ID NO: 3 - protein, 110 aa, Artificial Sequence
  C8-LC
QSALTQPASASGSPGQSVTISCTGTSSDVGGYNYVSWYQQHPGKAPKLMIYDVSKRPSGVSDRFSGSKSGNTASLTISGLQAEDGADYYCSSYRRGRTVVFGGGTKLTVL

SEQ ID NO: 4 - protein, 120 aa, Artificial Sequence
  C8-HC
QVQLQQWGGGLVQPGGSLRLSCAASGFTFSSYAMSWVRQAPGKGLEWVSAISGSGGSTYYADSVKGRFTISRDNSKNTLYLQMNSLRAEDTAVYYCAKNYFGNPRGFDYWGQGTMVTVSS

SEQ ID NO: 5 - protein, 107 aa, Artificial Sequence
  C11-LC
ETTLTQSPGTLSVSPGERVTLSCRASQSVSSYLAWYQQKPGQAPRLLIYGASTRATGIPDRFSGSGSGTDFTLTISRLEPEDFAVYYCQQYGISPLNFGGGTKVEIK

SEQ ID NO: 6 - protein, 126 aa, Artificial Sequence
  C11-HC
QVQLVQSGAEVKKPGSSVKVSCKASGGTFSSYAISWVRQAPGQGLEWMGGVIPIFGTANYAQKFRGRVTMTTDTSTSTAYMELRSLTSDDTAVYYCASPQGTWSTFLEWQGAFSVWGQGTTVTVSS

SEQ ID NO: 7 - protein, 115 aa, Artificial Sequence
  C14-LC
QAVLTQPSSLSASPGASVSLTCTLRSGINVGAYRVYWYQQKPGSPPQFLLRYKTDSDKQQGSGVPSRFSGSRDASANAGILLISGLRSEDEADYYCAIWHSSAWVFGGGTKVTVL

SEQ ID NO: 8 - protein, 122 aa, Artificial Sequence
  C14-HC
QVQLVQSGAEVKKPGASVKVSCKASGYTFTGYYMHWVRQAPGQGLEWMGRINPNSGGTNYAQKFQGRVTMTRDTSISTAYMELSRLRSDDTAVYYCARSPVWGSSRNWFDPWGQGTLVTVSS

SEQ ID NO: 9 - protein, 109 aa, Artificial Sequence
  C21-LC
GIVMTQSPATLSLSPGDRATLSCRASQSVSSSYLAWYQQKPGQAPRLLIYDASNRATGIPARFSGSGSGTDFTLTISSLEPEDFAVYYCQQRSNWPPITFGQGTKLEIK

SEQ ID NO: 10 - protein, 121 aa, Artificial Sequence
  C21-HC
QVQLVESGGGLVQPGGSLRLSCAASGFTFSSYAMSWVRQAPGKGLEWVSAISGSGGSTYYADSVKGRFTISRDNSKDTLYLQMNSLRAEDTAVYYCAKATTVVTPGYFDYWGQGTLVTVSS

SEQ ID NO: 11 - protein, 107 aa, Artificial Sequence
  C32-LC
DIQMTQSPAIMSASPGERVTMTCSASSSIRYIYWYQQKPGSSPRLLIYDTSNVAPGVPFRFSGSGSGTSYSLTINRMEAEDAATYYCQEWSGYPYTFGGGTKVEIKR

SEQ ID NO: 12 - protein, 121 aa, Artificial Sequence
  C32-HC
QVQLVQSGAEVKKPGSSVKVSCKASGGSFSSYAISWVRQAPGQGLEWMGGIIPIFGTANYAQKFQGRVTITADESTSTAYMELSSLRSEDTAVYYCANLRGGSSHYGMDVWGQGTLVTVSS

SEQ ID NO: 13 - DNA, 331 bp, Artificial Sequence
  C3-LC-g
cagtctgtgttgacgcagccgccctccgtgtctggggccccagggcagagggtcaccatctcctgcactgggagcagctccaacatcggggcagattatgatgtacactggtaccagcagcttccaggaacagcccccaaactcctcatctatggtaacaccaatcggccctcaggggtccctgaccgattctctggctccaagtctggcacctcagcctccctggccatcactgggctccaggctgaggatgaggctaattattactgccagtcctatgagagcggcctgggttggctgttcggcggagggacccagctcaccgttttag

SEQ ID NO: 14 - DNA, 364 bp, Artificial Sequence
  C3-HC-g
caggtgcagctggtggagtccgggggaggcttggtacagcctggggggtccctgagactctcctgtgcagcctctggattcacctttagcagctatgccatgagctgggtccgccaggctccagggaaggggctggagtgggtctcagctattagtggtagtggtggtagcacatactacgcagactccgtgaagggccggttcaccatctccagagacaattccaagaacacgctgtatctgcaaatgaacagcctgagagccgaggacacggccgtatattactgtgcgaaatacggtcggggactccccccaggacactttgactactggggccagggcaccctggtcaccgtctcctcag

SEQ ID NO: 15 - DNA, 331 bp, Artificial Sequence
  C8-LC-g
cagtctgccctgactcagcctgcctccgcgtccgggtctcctggacagtcagtcaccatctcctgcactggaaccagcagtgacgttggtggttataactatgtctcctggtaccaacagcacccaggcaaagcccccaaactcatgatttatgatgtgagcaagcgaccctcaggggtttctgatcgcttctctggctccaagtctggcaacacggcctccctgaccatctccgggctccaggctgaggacggggctgattattactgcagttcatatcgaaggggcaggactgtcgttttcggcggagggaccaagctgaccgtcctag

SEQ ID NO: 16 - DNA, 361 bp, Artificial Sequence
  C8-HC-g
caggtgcagctacagcagtgggggggaggcttggtacagcctggggggtccctgagactctcctgtgcagcctctggattcacctttagcagctatgccatgagctgggtccgccaggctccagggaaggggctggagtgggtctcagctattagtggtagtggtggtagcacatactacgcagactccgtgaagggccggttcaccatctccagagacaattccaagaacacgctgtatctgcaaatgaacagcctgagagccgaggacacggccgtatattactgtgcgaaaaactatttcgggaaccctaggggatttgactactggggccaggggacaatggtcaccgtctcctcag

SEQ ID NO: 17 - DNA, 322 bp, Artificial Sequence
  C11-LC-g
gaaacgacgctcacgcagtctccaggcaccctgtctgtgtctccaggggaaagagtcaccctctcctgtagggccagtcagagtgttagcagctacttagcctggtaccagcagaaacctggccaggctcccaggctcctcatctatggtgcatccaccagggccactggcatcccagacaggttcagtggcagtgggtctgggacagacttcactctcaccatcagcagactggagcctgaagattttgcagtgtattactgtcagcagtatggtatctcacctctcaatttcggcggggggaccaaagtggaaatcaaac

SEQ ID NO: 18 - DNA, 379 bp, Artificial Sequence
  C11-HC-g
caggtgcagctggtgcaatctggggctgaggtgaagaagcctgggtcctcggtgaaggtctcctgcaaggcttctggaggcaccttcagcagctatgctatcagctgggtgcgacaggcccctggacaagggcttgagtggatgggaggggtcatccctatctttggtacagcaaactacgcacagaagttccggggcagagtcaccatgaccacagacacatccacgagtacagcctacatggagctgaggagcctgacatctgacgacacggccgtgtattattgtgcgagtccccaaggcacgtggtcgacatttttggagtggcagggtgcttttagtgtctggggccaagggaccacggtcaccgtctcctcag

SEQ ID NO: 19 - DNA, 346 bp, Artificial Sequence
  C14-LC-g
caggctgtgctcactcagccgtcttccctctctgcatctcctggagcatcagtcagtctcacctgcactttacgcagtggcatcaatgttggtgcctacagggtatactggtaccagcagaagccagggagtcctccccagtttctcctgaggtacaaaacagactcagataagcagcagggctctggagtccccagccgcttctctggatccagagatgcttcggccaatgcagggattttactcatctctgggctccggtctgaggatgaggctgactattactgtgcgatttggcacagcagcgcttgggtgttcggcggagggaccaaggtcaccgtcctag

SEQ ID NO: 20 - DNA, 367 bp, Artificial Sequence
  C14-HC-g
caggttcagctggtacagtctggggctgaggtgaagaagcctggggcctcagtgaaggtctcctgcaaggcttctggatacaccttcaccggctactatatgcactgggtgcgacaggcccctggacaagggcttgagtggatggggcggatcaaccctaacagtggtggcacaaactatgcacagaagtttcagggcagggtcaccatgaccagggacacgtccatcagcacagcctacatggagctgagcaggctgagatctgacgacacggccgtgtattactgtgcgagaagccccgtgtggggatcaagcagaaactggttcgacccctggggccagggcaccctggtcaccgtctcctcag

SEQ ID NO: 21 - DNA, 328 bp, Artificial Sequence
  C21-LC-g
ggcatcgtgatgacccagtctccagccaccctatctttgtctccaggggatagagccaccctctcctgcagggccagtcagagtgttagcagcagctacttagcctggtaccagcagaaacctggccaggctcccaggctcctcatctatgatgcatccaacagggccactggcatcccagccaggttcagtggcagtgggtctgggacagacttcactctcaccatcagcagcctagagcctgaagattttgcagtttattactgtcagcaacgtagcaactggcctccgatcaccttcggccaagggaccaagctggagatcaaac

SEQ ID NO: 22 - DNA, 364 bp, Artificial Sequence
  C21-HC-g
caggtgcagctggtggagtctgggggaggcttggtacagcctggggggtccctgagactctcctgtgcagcctctggattcacctttagcagctatgccatgagctgggtccgccaggctccagggaaggggctggagtgggtctcagctattagtggtagtggtggtagcacatactacgcagactccgtgaagggccggttcaccatctccagagacaattccaaggacacgctgtatctgcaaatgaacagcctgagagccgaggacacggccgtatattactgtgcgaaagctactacggtggtaactccgggatactttgactactggggccagggcaccctggtcaccgtctcctcag

SEQ ID NO: 23 - DNA, 320 bp, Artificial Sequence
  C32-LC-g
gacatccagatgacccagtctccagcaatcatgtctgcatctccaggggagagggtcaccatgacctgcagtgccagctcaagtatacgttacatatattggtaccaacagaagcctggatcctcccccagactcctgatttatgacacatccaacgtggctcctggagtcccttttcgcttcagtggcagtgggtctgggacctcttattctctcacaatcaaccgaatggaggctgaggatgctgccacttattactgccaggagtggagtggttatccgtacacgttcggaggggggaccaaggtggagatcaaacg

SEQ ID NO: 24 - DNA, 363 bp, Artificial Sequence
  C32-HC-g
caggtgcagctggtgcaatctggggctgaggtgaagaagcctgggtcctcggtgaaggtctcctgcaaggcttctggaggctccttcagcagctatgctatcagctgggtgcgacaggcccctggacaagggcttgagtggatgggagggatcatccctatctttggtacagcaaactacgcacagaagttccagggcagagtcacgattaccgcggacgaatccacgagcacagcctacatggagctgagcagcctgagatctgaggacacggccgtgtattactgtgcgaaccttcggggtggtagctcccactacggtatggacgtctggggccagggaaccctggtcaccgtctcctca